European Patent Application EP 4 600 254 A1, published August 13, 2025. Title: 폐 기관지 특이적 유전자 전달이 가능한 아데노부속바이러스 벡터. Applicant: GluGene Therapeutics Inc. Application KR. The sequence listing filed with the application follows.

SEQUENCE LISTING (11 sequences)

SEQ ID NO: 1 - protein, 736 aa, Artificial Sequence
MAADGYLPDWLEDNLSEGIREWWDLKPGAPKPKANQQKQDDGRGLVLPGYKYLGPFNGLDKGEPVNAADAAALEHDKAYDQQLKAGDNPYLRYNHADAEFQERLQEDTSFGGNLGRAVFQAKKRVLEPLGLVEEGAKTAPGKKRPVEQSPQEPDSSSGIGKTGQQPAKKRLNFGQTGDSESVPDPQPLGEPPATPAAVGPTTMASGGGAPMADNNEGADGVGNASGNWHCDSTWLGDRVITTSTRTWALPTYNNHLYKQISSASTGASNDNHYFGYSTPWGYFDFNRFHCHFSPRDWQRLINNNWGFRPKRLNFKLFNIQVKEVTTNDGVTTIANNLTSTVQVFSDSEYQLPYVLGSAHQGCLPPFPADVFMIPQYGYLTLNNGSQAVGRSSFYCLEYFPSQMLRTGNNFTFSYTFEEVPFHSSYAHSQSLDRLMNPLIDQYLYYLNRTQNQSGSAQNKDLLFSRGSPAGMSVQPKNWLPGPCYRQQRVSKTKTDNNNSNFTWTGASKYNLNGRESIINPGTAMASHKDDEDKFFPMSGVMIFGKESAGASNTALDNVMITDEEEIKATNPVATERFGTVAVNFQSSSTDPATGDVHAMGALPGMVWQDRDVYLQGPIWAKIPHTDGHFHPSPLMGGFGLKNPPPQILIKNTPVPANPPAEFSATKFASFITQYSTGQVSVEIEWELQKENSKRWNPEVQYTSNYAKSANVDFTVDNNGLYTEPRPIGTRYLTRPL

SEQ ID NO: 2 - protein, 736 aa, Artificial Sequence
MAADGYLPDWLEDNLSEGIREWWDLKPGAPKPKANQQKQDDGRGLVLPGYKYLGPFNGLDKGEPVNAADAAALEHDKAYDQQLKAGDNPYLRYNHADAEFQERLQEDTSFGGNLGRAVFQAKKRVLEPLGLVEEGAKTAPGKKRPVEQSPQEPDSSSGIGKTGQQPAKKRLNFGQTGDSESVPDPQPLGEPPATPAAVGPTTMASGGGAPMADNNEGADGVGNASGNWHCDSTWLGDRVITTSTRTWALPTYNNHLYKQISSASTGASNDNHYFGYSTPWGYFDFNRFHCHFSPRDWQRLINNNWGFRPKRLNFKLFNIQVKEVTANDGVTTIANNLTSTVQVFSDSEYQLPYVLGSAHQGCLPPFPADVFMIPQYGYLTLNNGSQAVGRSSFYCLEYFPSQMLRTGNNFTFSYTFEEVPFHSSYAHSQSLDRLMNPLIDQYLYYLNRTQNPSGSAQNKDLLFSRGSPAGMSVQPKNWLPGPCYRQQRVSKTKTDNNNSNFTWTGASKYNLNGRESIINPGTAMASHKDDEDKFFPMSGVMIFGKESAGASNTALDNVMITDEEEIKATNPVATERFGTVAVNFQSSSTDPATGDVHAMGALPGMVWQDRDVYLQGPIWAKIPHTDGHFHPSPLMGGFGLKNPPPQILIKNTPVPANPPAEFSATKFASFITQYSTGQVSVEIEWELQKENSKRWNPEVQYTSNYAKSANVDFTVDNNGLYTEPRPIGTRYLTRPL

SEQ ID NO: 3 - protein, 736 aa, Artificial Sequence; identical to SEQ ID NO: 1

SEQ ID NO: 4 - DNA, 2205 bp, Artificial Sequence
  source 1..2205: mol_type = genomic DNA
atggctgccgatggttatcttccagattggctcgaggacaacctctctgagggcattcgcgagtggtgggacttgaaacctggagccccgaagcccaaagccaaccagcaaaagcaggacgacggccggggtctggtgcttcctggctacaagtacctcggacccttcaacggactcgacaagggggagcccgtcaacgcggcggacgcagcggccctcgagcacgacaaggcctacgaccagcagctcaaagcgggtgacaatccgtaccttcggtataaccacgccgacgccgagtttcaggagcgtctgcaagaagatacgtcttttgggggcaacctcgggcgagcagtcttccaggccaagaagcgggttctcgaacctctcggtctggttgaggaaggcgctaagacggctcctggaaagaaacgtccggtagagcagtcgccacaagagccagactcctcctcgggcatcggcaagacaggccagcagcccgctaaaaagagactcaattttggtcagactggcgactcagagtcagtccccgacccacaacctctcggagaacctccagcaacccccgctgctgtgggacctactacaatggcttcaggcggtggcgcaccaatggcagacaataacgaaggcgccgacggagtgggtaatgcctcaggaaattggcattgcgattccacatggctgggcgacagagtcatcaccaccagcacccgcacctgggccttgcccacctacaataaccacctctacaagcaaatctccagtgcttcaacgggggccagcaacgacaaccactacttcggctacagcaccccctgggggtattttgatttcaacagattccactgccacttttcaccacgtgactggcagcgactcatcaacaacaattggggattccggcccaagagactcaacttcaaactcttcaacatccaagtcaaggaggtcacgacgaatgatggcgtcacaaccatcgctaataaccttaccagcacggttcaagtcttctcggactcggagtaccagcttccgtacgtcctcggctctgcgcaccagggctgcctccctccgttcccggcggacgtgttcatgattccgcaatacggctacctgacgctcaacaatggcagccaagccgtgggacgttcatccttttactgcctggaatatttcccttctcagatgctgagaacgggcaacaactttaccttcagctacacctttgaggaagtgcctttccacagcagctacgcgcacagccagagcctggaccggctgatgaatcctctcatcgaccaatacctgtattacctgaacagaactcaaaatcagtccggaagtgcccaaaacaaggacttgctgtttagccgtgggtctccagctggcatgtctgttcagcccaaaaactggctacctggaccctgttatcggcagcagcgcgtttctaaaacaaaaacagacaacaacaacagcaattttacctggactggtgcttcaaaatataacctcaatgggcgtgaaaccatcatcaaccctggcactgctatggccaaagacgacgaagacaagttctttcccatgagcggtgtcatgatttttggaaaagagagcgccggagcttcaaacactgcattggacaatgtcatgattacagacgaagaggaaattaaagccactaaccctgtggccaccgaaagatttgggaccgtggcagtcgatttccagagcagcagcacagaccctgcgaccggagatgtgcatgctatgggagcattacctggcatggtgtggcaagatagagacgtgtacctgcagggtcccatttgggccaaaattcctcacacagatggacactttcacccgtctcctcttatgggcggctttggactcaagaacccgcctcctcagatcctcatcaaaaacacgcctgttcctgcgaatcctccggtggagttttcagctacaaagtttgcttcattcatcacccaatactccacaggacaagtgagtgtggaaattgaatgggagctgcagaaagaaaacagcaagcgctggaatcccgaagtgcagtacacatccaattatgcaaaatctgccaacgttgattttactgtggacaacaatggactttatactgagcctcgccccattggcacccgttaccttacccgtcccctgtaa

SEQ ID NO: 5 - DNA, 2205 bp, Artificial Sequence
  source 1..2205: mol_type = genomic DNA
atggctgccgatggttatcttccagattggctcgaggacaacctctctgagggcattcgcgagtggtgggacttgaaacctggagccccgaagcccaaagccaaccagcaaaagcaggacgacggccggggtctggtgcttcctggctacaagtacctcggacccttcaacggactcgacaagggggagcccgtcaacgcggcggacgcagcggccctcgagcacgacaaggcctacgaccagcagctcaaagcgggtgacaatccgtaccttcggtataaccacgccgacgccgagtttcaggagcgtctgcaagaagatacgtcttttgggggcaacctcgggcgagcagtcttccaggccaagaagcgggttctcgaacctctcggtctggttgaggaaggcgctaagacggctcctggaaagaaacgtccggtagagcagtcgccacaagagccagactcctcctcgggcatcggcaagacaggccagcagcccgctaaaaagagactcaattttggtcagactggcgactcagagtcagtccccgacccacaacctctcggagaacctccagcaacccccgctgctgtgggacctactacaatggcttcaggcggtggcgcaccaatggcagacaataacgaaggcgccgacggagtgggtaatgcctcaggaaattggcattgcgattccacatggctgggcgacagagtcatcaccaccagcacccgcacctgggccttgcccacctacaataaccacctctacaagcaaatctccagtgcttcaacgggggccagcaacgacaaccactacttcggctacagcaccccctgggggtattttgatttcaacagattccactgccacttttcaccacgtgactggcagcgactcatcaacaacaattggggattccggcccaagagactcaacttcaaactcttcaacatccaagtcaaggaggtcacgacgaatgatggcgtcacaaccatcgctaataaccttaccagcacggttcaagtcttctcggactcggagtaccagcttccgtacgtcctcggctctgcgcaccagggctgcctccctccgttcccggcggacgtgttcatgattccgcaatacggctacctgacgctcaacaatggcagccaagccgtgggacgttcatccttttactgcctggaatatttcccttctcagatgctgagaacgggcaacaactttaccttcagctacacctttgaggaagtgcctttccacagcagctacgcgcacagccagagcctggaccggctgatgaatcctctcatcgaccaatacctgtattacctgaacagaactcaaaatcagtccggaagtacccaaaacaaggacttgctgtttagccgtgggtctccagctggcatgtctgttcagcccaaaaactggctacctggaccctgttatcggcagcagcgcgtttctaaaacaaaaacagacaacaacaacagcaattttacctggactggtgcttcaaaatataacctcaatgggcgtgaaaccatcatcaaccctggcactgctatggccaaagacgacgaagacaagttctttcccatgagcggtgtcatgatttttggaaaagagagcgccggagcttcaaacactgcattggacaatgtcatgattacagacgaagaggaaattaaagccactaaccctgtggccaccgaaagatttgggaccgtggcagtcgatttccagagcagcagcacagaccctgcgaccggagatgtgcatgctatgggagcattacctggcatggtgtggcaagatagagacgtgtacctgcagggtcccatttgggccaaaattcctcacacagatggacactttcacccgtctcctcttatgggcggctttggactcaagaacccgcctcctcagatcctcatcaaaaacacgcctgttcctgcgaatcctccggtggagttttcagctacaaagtttgcttcattcatcacccaatactccacaggacaagtgagtgtggaaattgaatgggagctgcagaaagaaaacagcaagcgctggaatcccgaagtgcagtacacatccaattatgcaaaatctgccaacgttgattttactgtggacaacaatggactttatactgagcctcgccccattggcacccgttaccttacccgtcccctgtaa

SEQ ID NO: 6 - DNA, 7328 bp, Artificial Sequence
  source 1..7328: mol_type = genomic DNA
gcgcgccgatatcgttaacgccccgcgccggccgctctagaactagtggatcccccggaagatcagaagttcctattccgaagttcctattctctagaaagtataggaacttctgatctgcgcagccgccatgccggggttttacgagattgtgattaaggtccccagcgaccttgacgggcatctgcccggcatttctgacagctttgtgaactgggtggccgagaaggaatgggagttgccgccagattctgacatggatctgaatctgattgagcaggcacccctgaccgtggccgagaagctgcagcgcgactttctgacggaatggcgccgtgtgagtaaggccccggaggcccttttctttgtgcaatttgagaagggagagagctacttccacatgcacgtgctcgtggaaaccaccggggtgaaatccatggttttgggacgtttcctgagtcagattcgcgaaaaactgattcagagaatttaccgcgggatcgagccgactttgccaaactggttcgcggtcacaaagaccagaaatggcgccggaggcgggaacaaggtggtggatgagtgctacatccccaattacttgctccccaaaacccagcctgagctccagtgggcgtggactaatatggaacagtatttaagcgcctgtttgaatctcacggagcgtaaacggttggtggcgcagcatctgacgcacgtgtcgcagacgcaggagcagaacaaagagaatcagaatcccaattctgatgcgccggtgatcagatcaaaaacttcagccaggtacatggagctggtcgggtggctcgtggacaaggggattacctcggagaagcagtggatccaggaggaccaggcctcatacatctccttcaatgcggcctccaactcgcggtcccaaatcaaggctgccttggacaatgcgggaaagattatgagcctgactaaaaccgcccccgactacctggtgggccagcagcccgtggaggacatttccagcaatcggatttataaaattttggaactaaacgggtacgatccccaatatgcggcttccgtctttctgggatgggccacgaaaaagttcggcaagaggaacaccatctggctgtttgggcctgcaactaccgggaagaccaacatcgcggaggccatagcccacactgtgcccttctacgggtgcgtaaactggaccaatgagaactttcccttcaacgactgtgtcgacaagatggtgatctggtgggaggaggggaagatgaccgccaaggtcgtggagtcggccaaagccattctcggaggaagcaaggtgcgcgtggaccagaaatgcaagtcctcggcccagatagacccgactcccgtgatcgtcacctccaacaccaacatgtgcgccgtgattgacgggaactcaacgaccttcgaacaccagcagccgttgcaagaccggatgttcaaatttgaactcacccgccgtctggatcatgactttgggaaggtcaccaagcaggaagtcaaagactttttccggtgggcaaaggatcacgtggttgaggtggagcatgaattctacgtcaaaaagggtggagccaagaaaagacccgcccccagtgacgcagatataagtgagcccaaacgggtgcgcgagtcagttgcgcagccatcgacgtcagacgcggaagcttcgatcaactacgcagacaggtaccaaaacaaatgttctcgtcacgtgggcatgaatctgatgctgtttccctgcagacaatgcgagagaatgaatcagaattcaaatatctgcttcactcacggacagaaagactgtttagagtgctttcccgtgtcagaatctcaacccgtttctgtcgtcaaaaaggcgtatcagaaactgtgctacattcatcatatcatgggaaaggtgccagacgcttgcactgcctgcgatctggtcaatgtggatttggatgactgcatctttgaacaataaatgatttaaatcaggtatggctgccgatggttatcttccagattggctcgaggacaacctctctgagggcattcgcgagtggtgggacttgaaacctggagccccgaagcccaaagccaaccagcaaaagcaggacgacggccggggtctggtgcttcctggctacaagtacctcggacccttcaacggactcgacaagggggagcccgtcaacgcggcggacgcagcggccctcgagcacgacaaggcctacgaccagcagctcaaagcgggtgacaatccgtaccttcggtataaccacgccgacgccgagtttcaggagcgtctgcaagaagatacgtcttttgggggcaacctcgggcgagcagtcttccaggccaagaagcgggttctcgaacctctcggtctggttgaggaaggcgctaagacggctcctggaaagaaacgtccggtagagcagtcgccacaagagccagactcctcctcgggcatcggcaagacaggccagcagcccgctaaaaagagactcaattttggtcagactggcgactcagagtcagtccccgacccacaacctctcggagaacctccagcaacccccgctgctgtgggacctactacaatggcttcaggcggtggcgcaccaatggcagacaataacgaaggcgccgacggagtgggtaatgcctcaggaaattggcattgcgattccacatggctgggcgacagagtcatcaccaccagcacccgcacctgggccttgcccacctacaataaccacctctacaagcaaatctccagtgcttcaacgggggccagcaacgacaaccactacttcggctacagcaccccctgggggtattttgatttcaacagattccactgccacttttcaccacgtgactggcagcgactcatcaacaacaattggggattccggcccaagagactcaacttcaaactcttcaacatccaagtcaaggaggtcacggcgaatgatggcgtcacaaccatcgctaataaccttaccagcacggttcaagtcttctcggactcggagtaccagcttccgtacgtcctcggctctgcgcaccagggctgcctccctccgttcccggcggacgtgttcatgattccgcaatacggctacctgacgctcaacaatggcagccaagccgtgggacgttcatccttttactgcctggaatatttcccttctcagatgctgagaacgggcaacaactttaccttcagctacacctttgaggaagtgcctttccacagcagctacgcgcacagccagagcctggaccggctgatgaatcctctcatcgaccaatacctgtattacctgaacagaactcaaaatccgtccggaagtgcccaaaacaaggacttgctgtttagccgtgggtctccagctggcatgtctgttcagcccaaaaactggctacctggaccctgttatcggcagcagcgcgtttctaaaacaaaaacagacaacaacaacagcaattttacctggactggtgcttcaaaatataacctcaatgggcgtgaatccatcatcaaccctggcactgctatggcctcacacaaagacgacgaagacaagttctttcccatgagcggtgtcatgatttttggaaaagagagcgccggagcttcaaacactgcattggacaatgtcatgattacagacgaagaggaaattaaagccactaaccctgtggccaccgaaagatttgggaccgtggcagtcaatttccagagcagcagcacagaccctgcgaccggagatgtgcatgctatgggagcattacctggcatggtgtggcaagatagagacgtgtacctgcagggtcccatttgggccaaaattcctcacacagatggacactttcacccgtctcctcttatgggcggctttggactcaagaacccgcctcctcagatcctcatcaaaaacacgcctgttcctgcgaatcctccggcggagttttcagctacaaagtttgcttcattcatcacccaatactccacaggacaagtgagtgtggaaattgaatgggagctgcagaaagaaaacagcaagcgctggaatcccgaagtgcagtacacatccaattatgcaaaatctgccaacgttgattttactgtggacaacaatggactttatactgagcctcgccccattggcacccgttaccttacccgtcccctgtaattacgtgttaatcaataaaccggttaattcgtgtcagttgaactttggtctcatgtcgttattatcttatctggtcaccagatacgtagataagtagcatggcgggttaatcattaactacagcccgggcgtttaaacagcgggcggaggggtggagtcgtgacgtgaattacgtcatagggttagggaggtcctgtattagaggtcacgtgagtgttttgcgacattttgcgacaccatgtggtcacgctgggggggggggcccgagtgagcacgcagggtctccattttgaagcgggaggtttgaacgagcgctggcgcgctcactggccgtcgttttacaacgtcgtgactgggaaaaccctggcgttacccaacttaatcgccttgcagcacatccccctttcgccagctggcgtaatagcgaagaggcccgcaccgatcgcccttcccaacagttgcgcagcctgaatggcgaatgggtaaattgtaaacgttaatattttgttaaaattcgcgttaaatttttgttaaatcagctcattttttaaccaataggccgaaatcggcaaaatcccttataaatcaaaagaatagaccgagatagggttgagtgttgttccagtttggaacaagagtccactattaaagaacgtggactccaacgtcaaagggcgaaaaaccgtctatcagggcgatggcccactacgtgaaccatcaccctaatcaagttttttggggtcgaggtgccgtaaagcactaaatcggaaccctaaagggagcccccgatttagagcttgacggggaaagccggcgaacgtggcgagaaaggaagggaagaaagcgaaaggagcgggcgctagggcgctggcaagtgtagcggtcacgctgcgcgtaaccaccacacccgccgcgcttaatgcgccgctacagggcgcgtggtggcacttttcggggaaatgtgcgcggaacccctatttgtttatttttctaaatacattcaaatatgtatccgctcatgagacaataaccctgataaatgcttcaataatattgaaaaaggaagagtatgagtattcaacatttccgtgtcgcccttattcccttttttgcggcattttgccttcctgtttttgctcacccagaaacgctggtgaaagtaaaagatgctgaagatcagttgggtgcacgagtgggttacatcgaactggatctcaacagcggtaagatccttgagagttttcgccccgaagaacgttttccaatgatgagcacttttaaagttctgctatgtggcgcggtattatcccgtattgacgccgggcaagagcaactcggtcgccgcatacactattctcagaatgacttggttgagtactcaccagtcacagaaaagcatcttacggatggcatgacagtaagagaattatgcagtgctgccataagcatgagtgataacactgcggccaacttacttctgacaacgatcggaggaccgaaggagctaaccgctttttttcacaacatgggggatcatgtaactcgccttgatcgttgggaaccggagctgaatgaagccataccaaacgacgagcgtgacaccacgatgcctgtagcaatggcaacaacgttgcgcaaactattaactggcgaactacttactctagcttcccggcaacaattaatagactggatggaggcggataaagttgcaggaccacttctgcgctcggcccttccggctggctggtttattgctgataaatctggagccggtgagcgtgggtctcgcggtatcattgcagcactggggccagatggtaagccctcccgtatcgtagttatctacacgacgggcagtcaggcaactatggatgaacgaaatagacagatcgctgagataggtgcctcactgattaagcattggtaactgtcagaccaagtttactcatatatactttagattgatttaaaacttcatttttaatttaaaaggatctaggtgaagatcctttttgataatctcatgaccaaaatcccttaacgtgagttttcgttccactgagcgtcagaccccgtagaaaagatcaaaggatcttcttgagatcctttttttctgcgcgtaatctgctgcttgcaaacaaaaaaaccaccgctaccagcggtggtttgtttgccggatcaagagctaccaactctttttccgaaggtaactggcttcagcagagcgcagataccaaatactgtccttctagtgtagccgtagttaggccaccacttcaagaactctgtagcaccgcctacatacctcgctctgctaatcctgttaccagtggctgctgccagtggcgataagtcgtgtcttaccgggttggactcaagacgatagttaccggataaggcgcagcggtcgggctgaacggggggttcgtgcacacagcccagcttggagcgaacgacctacaccgaactgagatacctacagcgtgagcattgagaaagcgccacgcttcccgaagggagaaaggcggacaggtatccggtaagcggcagggtcggaacaggagagcgcacgagggagcttccaggggggaacgcctggtatctttatagtcctgtcgggtttcgccacctctgacttgagcgtcgatttttgtgatgctcgtcaggggggccgagcctatggaaaaacgccagcaacgcggcctttttacggttcctggccttttgctggccttttgctcacatgttctttcctgcgttatcccctgattctgtggataaccgtattaccgcctttgagtgagctgataccgctcgccgcagccgaacgaccgagcgcagcgagtcagtgagcgaggaagcggaagagcgcccaatacgcaaaccgcctctccccgcgcgttggccgattcattaatgcagctggcacgacaggtttcccgactggaaagcgggcagtgagcgcaacgcaattaatgtgagttacctcactcattaggcaccccaggctttacactttatgcttccggctcctatgttgtgtggaattgtgagcggataacaatttcacacaggaaacagctatgaccatgattacgccaa

SEQ ID NO: 7 - DNA, 7328 bp, Artificial Sequence
  source 1..7328: mol_type = genomic DNA
gcgcgccgatatcgttaacgccccgcgccggccgctctagaactagtggatcccccggaagatcagaagttcctattccgaagttcctattctctagaaagtataggaacttctgatctgcgcagccgccatgccggggttttacgagattgtgattaaggtccccagcgaccttgacgggcatctgcccggcatttctgacagctttgtgaactgggtggccgagaaggaatgggagttgccgccagattctgacatggatctgaatctgattgagcaggcacccctgaccgtggccgagaagctgcagcgcgactttctgacggaatggcgccgtgtgagtaaggccccggaggcccttttctttgtgcaatttgagaagggagagagctacttccacatgcacgtgctcgtggaaaccaccggggtgaaatccatggttttgggacgtttcctgagtcagattcgcgaaaaactgattcagagaatttaccgcgggatcgagccgactttgccaaactggttcgcggtcacaaagaccagaaatggcgccggaggcgggaacaaggtggtggatgagtgctacatccccaattacttgctccccaaaacccagcctgagctccagtgggcgtggactaatatggaacagtatttaagcgcctgtttgaatctcacggagcgtaaacggttggtggcgcagcatctgacgcacgtgtcgcagacgcaggagcagaacaaagagaatcagaatcccaattctgatgcgccggtgatcagatcaaaaacttcagccaggtacatggagctggtcgggtggctcgtggacaaggggattacctcggagaagcagtggatccaggaggaccaggcctcatacatctccttcaatgcggcctccaactcgcggtcccaaatcaaggctgccttggacaatgcgggaaagattatgagcctgactaaaaccgcccccgactacctggtgggccagcagcccgtggaggacatttccagcaatcggatttataaaattttggaactaaacgggtacgatccccaatatgcggcttccgtctttctgggatgggccacgaaaaagttcggcaagaggaacaccatctggctgtttgggcctgcaactaccgggaagaccaacatcgcggaggccatagcccacactgtgcccttctacgggtgcgtaaactggaccaatgagaactttcccttcaacgactgtgtcgacaagatggtgatctggtgggaggaggggaagatgaccgccaaggtcgtggagtcggccaaagccattctcggaggaagcaaggtgcgcgtggaccagaaatgcaagtcctcggcccagatagacccgactcccgtgatcgtcacctccaacaccaacatgtgcgccgtgattgacgggaactcaacgaccttcgaacaccagcagccgttgcaagaccggatgttcaaatttgaactcacccgccgtctggatcatgactttgggaaggtcaccaagcaggaagtcaaagactttttccggtgggcaaaggatcacgtggttgaggtggagcatgaattctacgtcaaaaagggtggagccaagaaaagacccgcccccagtgacgcagatataagtgagcccaaacgggtgcgcgagtcagttgcgcagccatcgacgtcagacgcggaagcttcgatcaactacgcagacaggtaccaaaacaaatgttctcgtcacgtgggcatgaatctgatgctgtttccctgcagacaatgcgagagaatgaatcagaattcaaatatctgcttcactcacggacagaaagactgtttagagtgctttcccgtgtcagaatctcaacccgtttctgtcgtcaaaaaggcgtatcagaaactgtgctacattcatcatatcatgggaaaggtgccagacgcttgcactgcctgcgatctggtcaatgtggatttggatgactgcatctttgaacaataaatgatttaaatcaggtatggctgccgatggttatcttccagattggctcgaggacaacctctctgagggcattcgcgagtggtgggacttgaaacctggagccccgaagcccaaagccaaccagcaaaagcaggacgacggccggggtctggtgcttcctggctacaagtacctcggacccttcaacggactcgacaagggggagcccgtcaacgcggcggacgcagcggccctcgagcacgacaaggcctacgaccagcagctcaaagcgggtgacaatccgtaccttcggtataaccacgccgacgccgagtttcaggagcgtctgcaagaagatacgtcttttgggggcaacctcgggcgagcagtcttccaggccaagaagcgggttctcgaacctctcggtctggttgaggaaggcgctaagacggctcctggaaagaaacgtccggtagagcagtcgccacaagagccagactcctcctcgggcatcggcaagacaggccagcagcccgctaaaaagagactcaattttggtcagactggcgactcagagtcagtccccgacccacaacctctcggagaacctccagcaacccccgctgctgtgggacctactacaatggcttcaggcggtggcgcaccaatggcagacaataacgaaggcgccgacggagtgggtaatgcctcaggaaattggcattgcgattccacatggctgggcgacagagtcatcaccaccagcacccgcacctgggccttgcccacctacaataaccacctctacaagcaaatctccagtgcttcaacgggggccagcaacgacaaccactacttcggctacagcaccccctgggggtattttgatttcaacagattccactgccacttttcaccacgtgactggcagcgactcatcaacaacaattggggattccggcccaagagactcaacttcaaactcttcaacatccaagtcaaggaggtcacgacgaatgatggcgtcacaaccatcgctaataaccttaccagcacggttcaagtcttctcggactcggagtaccagcttccgtacgtcctcggctctgcgcaccagggctgcctccctccgttcccggcggacgtgttcatgattccgcaatacggctacctgacgctcaacaatggcagccaagccgtgggacgttcatccttttactgcctggaatatttcccttctcagatgctgagaacgggcaacaactttaccttcagctacacctttgaggaagtgcctttccacagcagctacgcgcacagccagagcctggaccggctgatgaatcctctcatcgaccaatacctgtattacctgaacagaactcaaaatcagtccggaagtacccaaaacaaggacttgctgtttagccgtgggtctccagctggcatgtctgttcagcccaaaaactggctacctggaccctgttatcggcagcagcgcgtttctaaaacaaaaacagacaacaacaacagcaattttacctggactggtgcttcaaaatataacctcaatgggcgtgaatccatcatcaaccctggcactgctatggcctcacacaaagacgacgaagacaagttctttcccatgagcggtgtcatgatttttggaaaagagagcgccggagcttcaaacactgcattggacaatgtcatgattacagacgaagaggaaattaaagccactaaccctgtggccaccgaaagatttgggaccgtggcagtcaatttccagagcagcagcacagaccctgcgaccggagatgtgcatgctatgggagcattacctggcatggtgtggcaagatagagacgtgtacctgcagggtcccatttgggccaaaattcctcacacagatggacactttcacccgtctcctcttatgggcggctttggactcaagaacccgcctcctcagatcctcatcaaaaacacgcctgttcctgcgaatcctccggcggagttttcagctacaaagtttgcttcattcatcacccaatactccacaggacaagtgagtgtggaaattgaatgggagctgcagaaagaaaacagcaagcgctggaatcccgaagtgcagtacacatccaattatgcaaaatctgccaacgttgattttactgtggacaacaatggactttatactgagcctcgccccattggcacccgttaccttacccgtcccctgtaattacgtgttaatcaataaaccggttaattcgtgtcagttgaactttggtctcatgtcgttattatcttatctggtcaccagatacgtagataagtagcatggcgggttaatcattaactacagcccgggcgtttaaacagcgggcggaggggtggagtcgtgacgtgaattacgtcatagggttagggaggtcctgtattagaggtcacgtgagtgttttgcgacattttgcgacaccatgtggtcacgctgggggggggggcccgagtgagcacgcagggtctccattttgaagcgggaggtttgaacgagcgctggcgcgctcactggccgtcgttttacaacgtcgtgactgggaaaaccctggcgttacccaacttaatcgccttgcagcacatccccctttcgccagctggcgtaatagcgaagaggcccgcaccgatcgcccttcccaacagttgcgcagcctgaatggcgaatgggtaaattgtaaacgttaatattttgttaaaattcgcgttaaatttttgttaaatcagctcattttttaaccaataggccgaaatcggcaaaatcccttataaatcaaaagaatagaccgagatagggttgagtgttgttccagtttggaacaagagtccactattaaagaacgtggactccaacgtcaaagggcgaaaaaccgtctatcagggcgatggcccactacgtgaaccatcaccctaatcaagttttttggggtcgaggtgccgtaaagcactaaatcggaaccctaaagggagcccccgatttagagcttgacggggaaagccggcgaacgtggcgagaaaggaagggaagaaagcgaaaggagcgggcgctagggcgctggcaagtgtagcggtcacgctgcgcgtaaccaccacacccgccgcgcttaatgcgccgctacagggcgcgtggtggcacttttcggggaaatgtgcgcggaacccctatttgtttatttttctaaatacattcaaatatgtatccgctcatgagacaataaccctgataaatgcttcaataatattgaaaaaggaagagtatgagtattcaacatttccgtgtcgcccttattcccttttttgcggcattttgccttcctgtttttgctcacccagaaacgctggtgaaagtaaaagatgctgaagatcagttgggtgcacgagtgggttacatcgaactggatctcaacagcggtaagatccttgagagttttcgccccgaagaacgttttccaatgatgagcacttttaaagttctgctatgtggcgcggtattatcccgtattgacgccgggcaagagcaactcggtcgccgcatacactattctcagaatgacttggttgagtactcaccagtcacagaaaagcatcttacggatggcatgacagtaagagaattatgcagtgctgccataagcatgagtgataacactgcggccaacttacttctgacaacgatcggaggaccgaaggagctaaccgctttttttcacaacatgggggatcatgtaactcgccttgatcgttgggaaccggagctgaatgaagccataccaaacgacgagcgtgacaccacgatgcctgtagcaatggcaacaacgttgcgcaaactattaactggcgaactacttactctagcttcccggcaacaattaatagactggatggaggcggataaagttgcaggaccacttctgcgctcggcccttccggctggctggtttattgctgataaatctggagccggtgagcgtgggtctcgcggtatcattgcagcactggggccagatggtaagccctcccgtatcgtagttatctacacgacgggcagtcaggcaactatggatgaacgaaatagacagatcgctgagataggtgcctcactgattaagcattggtaactgtcagaccaagtttactcatatatactttagattgatttaaaacttcatttttaatttaaaaggatctaggtgaagatcctttttgataatctcatgaccaaaatcccttaacgtgagttttcgttccactgagcgtcagaccccgtagaaaagatcaaaggatcttcttgagatcctttttttctgcgcgtaatctgctgcttgcaaacaaaaaaaccaccgctaccagcggtggtttgtttgccggatcaagagctaccaactctttttccgaaggtaactggcttcagcagagcgcagataccaaatactgtccttctagtgtagccgtagttaggccaccacttcaagaactctgtagcaccgcctacatacctcgctctgctaatcctgttaccagtggctgctgccagtggcgataagtcgtgtcttaccgggttggactcaagacgatagttaccggataaggcgcagcggtcgggctgaacggggggttcgtgcacacagcccagcttggagcgaacgacctacaccgaactgagatacctacagcgtgagcattgagaaagcgccacgcttcccgaagggagaaaggcggacaggtatccggtaagcggcagggtcggaacaggagagcgcacgagggagcttccaggggggaacgcctggtatctttatagtcctgtcgggtttcgccacctctgacttgagcgtcgatttttgtgatgctcgtcaggggggccgagcctatggaaaaacgccagcaacgcggcctttttacggttcctggccttttgctggccttttgctcacatgttctttcctgcgttatcccctgattctgtggataaccgtattaccgcctttgagtgagctgataccgctcgccgcagccgaacgaccgagcgcagcgagtcagtgagcgaggaagcggaagagcgcccaatacgcaaaccgcctctccccgcgcgttggccgattcattaatgcagctggcacgacaggtttcccgactggaaagcgggcagtgagcgcaacgcaattaatgtgagttacctcactcattaggcaccccaggctttacactttatgcttccggctcctatgttgtgtggaattgtgagcggataacaatttcacacaggaaacagctatgaccatgattacgccaa

SEQ ID NO: 8 - DNA, 22 bp, Artificial Sequence
  source 1..22: mol_type = unassigned DNA
gcggaagcttcgatcaactacg

SEQ ID NO: 9 - DNA, 23 bp, Artificial Sequence
  source 1..23: mol_type = unassigned DNA
cgcagagaccaaagttcaactga

SEQ ID NO: 10 - DNA, 21 bp, Artificial Sequence
  source 1..21: mol_type = unassigned DNA
atggtgatgcggttttggcag

SEQ ID NO: 11 - DNA, 24 bp, Artificial Sequence
  source 1..24: mol_type = unassigned DNA
ggcggagttgttacgacattttgg